European Patent Specification EP 3 725 333 B1, published August 23, 2023. Title: Peptide Sequence Design and Use Thereof for Peptide-Mediated siRNA Delivery. Applicant: CHEN, Pu JAFARI, Mousa XU, Wen CHEN, Baoling PAN, Ran KARUNARATNE, Nedra. Application PCT. The sequence listing filed with the application follows.

SEQUENCE LISTING (50 sequences)

SEQ ID NO: 1 - protein, 18 aa, Artificial Sequence
  C1M
FQFNFQFNGGGPKKKRKV

SEQ ID NO: 2 - protein, 18 aa, Artificial Sequence
  C1M1
FQFNFQFNGGGPKPKRKV

SEQ ID NO: 3 - protein, 22 aa, Artificial Sequence
  C1M2
FQFNFQFNFQFNGGGPKKKRKV

SEQ ID NO: 4 - protein, 22 aa, Artificial Sequence
  C1M3
FQFNFQFNFQFNWSQPKPKRKV

SEQ ID NO: 5 - protein, 22 aa, Artificial Sequence
  C1M4
FQFNFQFNFQFNGGGPKPKRKV

SEQ ID NO: 6 - protein, 26 aa, Artificial Sequence
  C1M5
FQFNFQFNFQFNGGGCHHRRRRRRHC

SEQ ID NO: 7 - protein, 24 aa, Artificial Sequence
  C1M6
FQFNFQFNFQFNGGGCPKPKRKVC

SEQ ID NO: 8 - protein, 15 aa, Artificial Sequence
  E3M
RLTLHLRLELTLHLE

SEQ ID NO: 9 - protein, 15 aa, Artificial Sequence
  E3M1
RWTWHWRWEWTWHWE

SEQ ID NO: 10 - protein, 21 aa, Artificial Sequence
  A7M
RHALAHLLHKLKHLLHALAHR

SEQ ID NO: 11 - protein, 21 aa, Artificial Sequence
  A7M1
RHALAHLLHRLRHLLHALAHR

SEQ ID NO: 12 - protein, 18 aa, Artificial Sequence
  C6M
RLWRLWLRLWRRLWRLLR

SEQ ID NO: 13 - protein, 18 aa, Artificial Sequence
  C6M1
RLWRLLWRLWRRLWRLLR

SEQ ID NO: 14 - protein, 18 aa, Artificial Sequence
  C6M2
RLWRLLWHLWRHLWRLLR

SEQ ID NO: 15 - protein, 18 aa, Artificial Sequence
  C6M3
RLWHLLWRLWRRLHRLLR

SEQ ID NO: 16 - protein, 18 aa, Artificial Sequence
  C6M4
HLLRLLLRLWHRLWRLLR

SEQ ID NO: 17 - protein, 18 aa, Artificial Sequence
  C6M5
HLWHLLLRLWRRLLRLLR

SEQ ID NO: 18 - protein, 18 aa, Artificial Sequence
  C6M6
GLWHLLLHLWRRLLRLLR

SEQ ID NO: 19 - protein, 18 aa, Artificial Sequence
  C6M7
GLWHLLLHLWRRHHRHHR

SEQ ID NO: 20 - protein, 18 aa, Artificial Sequence
  C6M8
GLWHLHLHLWRRHHRLLR

SEQ ID NO: 21 - protein, 18 aa, Artificial Sequence
  C6M9
GLWHLLLHLWHRLLRHHR

SEQ ID NO: 22 - protein, 24 aa, Artificial Sequence
  MW1
MWKSKIGSWILVRWAMWSKKRPKP

SEQ ID NO: 23 - protein, 24 aa, Artificial Sequence
  MW2
MWKSHIGSWILVRWAMWSHKRPKP

SEQ ID NO: 24 - protein, 23 aa, Artificial Sequence
  MW3
MWKSKISWILVSKPGLCKKRPKP

SEQ ID NO: 25 - protein, 23 aa, Artificial Sequence
  MW4
MHKSKISWHLVSKPGLCHKRPKP

SEQ ID NO: 26 - protein, 18 aa, Artificial Sequence
  C6-Dr
RLLRLLLRLWRRLLRLLR

SEQ ID NO: 27 - protein, 18 aa, Artificial Sequence
  C6-D
RLLRLLLRLWRRLLRLLR

SEQ ID NO: 28 - protein, 18 aa, Artificial Sequence
  C6M1-Dr
RLWRLLWRLWRRLWRLLR

SEQ ID NO: 29 - protein, 18 aa, Artificial Sequence
  C6M1-D
RLWRLLWRLWRRLWRLLR

SEQ ID NO: 30 - protein, 18 aa, Artificial Sequence
  C6M3-Dr
RLWHLLWRLWRRLHRLLR

SEQ ID NO: 31 - protein, 18 aa, Artificial Sequence
  C6M3-D
RLWHLLWRLWRRLHRLLR

SEQ ID NO: 32 - protein, 18 aa, Artificial Sequence
  C6M6-Dr
GLWHLLLHLWRRLLRLLR

SEQ ID NO: 33 - protein, 18 aa, Artificial Sequence
  C6M6-D
GLWHLLLHLWRRLLRLLR

SEQ ID NO: 34 - protein, 24 aa, Artificial Sequence
  GL1
GLWRAWLWKAFLASNWRRLLRLLR

SEQ ID NO: 35 - protein, 24 aa, Artificial Sequence
  GL2
GLWRASWLKAWLASNWHKKHRLLR

SEQ ID NO: 36 - protein, 25 aa, Artificial Sequence
  GL3
GLWGAWFIEGWEGMIDGRRLLRLLR

SEQ ID NO: 37 - protein, 23 aa, Artificial Sequence
  GL4
GLWRASWLKAFLASNWHKKLHKK

SEQ ID NO: 38 - protein, 38 aa, Artificial Sequence
  HA2-C6
GLFGAIAGFIENGWEGMIDGRLLRLLLRLWRRLLRLLR

SEQ ID NO: 39 - protein, 30 aa, Artificial Sequence
  HA2-PK
GLFGAIAGFIENGWEGMIDGWYGPKKKRKV

SEQ ID NO: 40 - protein, 10 aa, Artificial Sequence
  STR-C1
  MISC_FEATURE (1)..(1): STR modified sequence
GGGPKPKRKV

SEQ ID NO: 41 - protein, 10 aa, Artificial Sequence
  STR-HK
  MISC_FEATURE (1)..(1): STR modified sequence
HHHPKPKRKV

SEQ ID NO: 42 - protein, 12 aa, Artificial Sequence
  STR-HKC
  MISC_FEATURE (1)..(1): STR modified sequence
HHHCPKKKRKVC

SEQ ID NO: 43 - protein, 18 aa, Artificial Sequence
  C6-CYSt
  MISC_FEATURE (18)..(18): CYSt modified sequence
RLLRLLLRLWRRLLRLLR

SEQ ID NO: 44 - protein, 18 aa, Artificial Sequence
  C6M1-CYSt
  MISC_FEATURE (18)..(18): CYSt modified sequence
RLWRLLWRLWRRLWRLLR

SEQ ID NO: 45 - protein, 18 aa, Artificial Sequence
  C6M3-CYSt
  MISC_FEATURE (18)..(18): CYSt modified sequence
RLWHLLWRLWRRLHRLLR

SEQ ID NO: 46 - protein, 18 aa, Artificial Sequence
  C6M6-CYSt
  MISC_FEATURE (18)..(18): CYSt modified sequence
GLWHLLLHLWRRLLRLLR

SEQ ID NO: 47 - DNA, 21 bp, Artificial Sequence
  Primer 1
ttgctgttgaagtcgcaggag

SEQ ID NO: 48 - DNA, 20 bp, Artificial Sequence
  Primer 2
tgtgtccgtcgtggatctga

SEQ ID NO: 49 - DNA, 24 bp, Artificial Sequence
  Primer 3
agggtttctccacttcgatcttgc

SEQ ID NO: 50 - DNA, 24 bp, Artificial Sequence
  Primer 4
agatggcacaggaggaaagagcat